European Patent Application EP 4 190 343 A1, published June 7, 2023. Title: Peptides and pharmaceutical, nutraceutical or veterinary compositions for hair loss prevention and/or treatment. Applicant: VYTRUS BIOTECH, S.L. The sequence listing filed with the application follows.

SEQUENCE LISTING (19 sequences)

SEQ ID NO: 1 - protein, 5 aa, synthetic construct
  MOD_RES 1: note = ACYLATION - Acylated N-terminal tyrosine with R1 radical, wherein R1 is a -C(O)-(C1-C20)-alkyl radical; note = N-terminal tyrosine with the side-chain hydroxyl group optionally replaced by a radical -OSO3R3; being R3 selected from H and (C1-C3)-alkyl
  MOD_RES 3: note = Tyrosine with the side-chain hydroxyl group optionally replaced by a radical -OSO3R3; being R3 selected from H and (C1-C3)-alkyl
  MOD_RES 4: note = AMIDATION - Amidated C-terminal threonine with a R2 radical, when in formula (I) p is 0, and wherein R2 is a -NR4R5 radical, being R4 and R5 selected from H, and (C1-C3)-alkyl
  MOD_RES 5: note = AMIDATION - Amidated C-terminal glutamine with a R2 radical, when in formula (I) p is 1, and wherein R2 is a -NR4R5 radical, being R4 and R5 selected from H, and (C1-C3)-alkyl
YIYTQ

SEQ ID NO: 2 - protein, 4 aa, synthetic construct
  MOD_RES 1: note = ACETYLATION - Acetylated N-terminal Tyrosine; note = SULFATATION - Tyrosine (Y) sulphated with a radical -OSO3H
  MOD_RES 4: note = AMIDATION - Amidated C-terminal Threonine
YIYT

SEQ ID NO: 3 - protein, 4 aa, synthetic construct
  MOD_RES 1: note = ACETYLATION - Acetylated N-terminal Tyrosine
  MOD_RES 3: note = SULFATATION - Tyrosine (Y) sulphated with a radical -OSO3H.
  MOD_RES 4: note = AMIDATION - Amidated C-terminal Threonine
YIYT

SEQ ID NO: 4 - protein, 5 aa, synthetic construct
  MOD_RES 1: note = ACETYLATION - Acetylated N-terminal Tyrosine
  MOD_RES 1: note = SULFATATION - Tyrosine (Y) sulphated with a radical -OSO3H
  MOD_RES 5: note = AMIDATION - Amidated C-terminal Glutamine
YIYTQ

SEQ ID NO: 5 - protein, 5 aa, synthetic construct
  MOD_RES 1: note = ACETYLATION - Acetylated N-terminal Tyrosine
  MOD_RES 3: note = SULFATATION - Tyrosine (Y) sulphated with a radical -OSO3H
  MOD_RES 3: note = AMIDATION - Amidated C-terminal Glutamine
YIYTQ

SEQ ID NO: 6 - protein, 4 aa, synthetic construct
  MOD_RES 1: note = ACETYLATION - Acetylated N-terminal Tyrosine
  MOD_RES 4: note = AMIDATION - Amidated C-terminal Threonine
YIYT

SEQ ID NO: 7 - protein, 5 aa, synthetic construct
  MOD_RES 1: note = ACETYLATION - Acetylated N-terminal Tyrosine
  MOD_RES 5: note = AMIDATION - Amidated C-terminal Glutamine
YIYTQ

SEQ ID NO: 8 - protein, 4 aa, synthetic construct
  MOD_RES 1: note = SULFATATION - Tyrosine (Y) sulphated with a radical -OSO3H
YIYT

SEQ ID NO: 9 - protein, 4 aa, synthetic construct
  MOD_RES 3: note = SULFATATION - Tyrosine (Y) sulphated with a radical -OSO3H
YIYT

SEQ ID NO: 10 - protein, 5 aa, synthetic construct
  REGION 1..5: note = Synthetic peptide
  MOD_RES 1: note = SULFATATION - Tyrosine (Y) sulphated with a radical -OSO3H
YIYTQ

SEQ ID NO: 11 - protein, 5 aa, synthetic construct
  MOD_RES 3: note = SULFATATION - Tyrosine (Y) sulphated with a radical -OSO3H
YIYTQ

SEQ ID NO: 12 - protein, 4 aa, synthetic construct
YIYT

SEQ ID NO: 13 - protein, 5 aa, synthetic construct
YIYTQ

SEQ ID NO: 14 - protein, 4 aa, synthetic construct
  MOD_RES 1: note = SULFATATION - Tyrosine (Y) sulphated with a radical -OSO3H
  MOD_RES 3: note = SULFATATION - Tyrosine (Y) sulphated with a radical -OSO3H
YIYT

SEQ ID NO: 15 - protein, 5 aa, synthetic construct
  MOD_RES 1: note = SULFATATION - Tyrosine (Y) sulphated with a radical -OSO3H
  MOD_RES 3: note = SULFATATION - Tyrosine (Y) sulphated with a radical -OSO3H
YIYTQ

SEQ ID NO: 16 - protein, 4 aa, synthetic construct
  MOD_RES 1: note = ACETYLATION - Acetylated N-terminal Tyrosine
YIYT

SEQ ID NO: 17 - protein, 5 aa, synthetic construct
  MOD_RES 1: note = ACETYLATION - Acetylated N-terminal Tyrosine
YIYTQ

SEQ ID NO: 18 - protein, 4 aa, synthetic construct
  MOD_RES 4: note = AMIDATION - Amidated C-terminal Threonine
YIYT

SEQ ID NO: 19 - protein, 5 aa, synthetic construct
  MOD_RES 5: note = AMIDATION - Amidated C-terminal Glutamine
YIYTQ